European Patent Application EP 4 265 718 A1, published October 25, 2023. Title: NOVEL SINGLE-SUBUNIT RNA POLYMERASE. Applicant: UNIVERSITAET HAMBURG. The sequence listing filed with the application follows.

SEQUENCE LISTING (15 sequences)

SEQ ID NO: 1 - protein, 816 aa, Unknown
  single-subunit RNA polymerase
MHYETLEQKVERQIQLEKDYRTRSLNKSRELVQKAMQAGNLSSLPKVSRMIAAAYDTVAAGIDAMKAEKTAGVGGKYRSIIRLVPTDVLAVMTLTKCFDALFVSEGGSSRVSAGTLLANIGRQVQAEVLAIQLETVAPAYMNRVFEYLKERNTTSPSHIMKTLRASAENVHLGHEPWSNSQCVSVGKLLLQPAWDTGLFTWDKATDATRMSYLAPSEELAEHLQELVEDADTVDIKPPMLVKPNRHETLFSGGYLLPSTCKRGTYHNRQITRAMKRDVAEAFKSADQVKEALNKSQEVAYVINKEVLALINEARRSGVATGMPSSYPAPKPEWYLDGVPKEEYTERQMGDFQTWKMNMRNWYINERARVSKLRSLVSLTQICEEFKDESELYFPTCVDWRYRLYFKSSLHPQGSDMQKALLSFAKAKPLGERGLFWLKVHVATCYGYDKALFEKRAAWTDDNIQQVREVARAPFNAEAFKSADAPWCFLAACIDLVNAFDSESPELYESRIPVAMDATNSGSQHFSALLRDPVGGKLTNLFWEGNEEKADMYMDVKQRTDSKVIMDLDNPEFVVQAQFWRENEITRSMTKRPCMTHVYSATVRSCSEYILQSAQEEGYEGTEEYSLFKLAGYLSGRMKSAVEDANPAATAAMKYLQSLCYRVPAANHLEWKTPLGALVINRYTESEETKVAVRSMNISQLLIYNRNYDVNNKRKAKSGISPNWIHSLDATHLMMTINAFEGDIMPIHDSVATHACDVDAMHAAVREQFVRLYTEHDVLEEITDAAVKCGADLEGLEMPVKGALDIKQVVKSPFFFC

SEQ ID NO: 2 - DNA, 18 bp, Unknown
  Promoter e
tcagaagtcacactataa

SEQ ID NO: 3 - DNA, 18 bp, Unknown
  Promoter f
aatagaaacatactataa

SEQ ID NO: 4 - DNA, 18 bp, SP6-like viruses
  Promoter b
aatagaaacatactataa

SEQ ID NO: 5 - DNA, 47 bp, Artificial Sequence
  Primer
  promoter 10..27: /note="promoter a"
ataagatctaattaaccctcactaaaggggaattgtgagcggataac

SEQ ID NO: 6 - DNA, 47 bp, Artificial Sequence
  Primer
  promoter 10..27: /note="promoter b"
ataagatctatttaggtgacactataggggaattgtgagcggataac

SEQ ID NO: 7 - DNA, 47 bp, Artificial Sequence
  Primer
  promoter 10..27: /note="promoter c"
ataagatcttaatacgactcactataggggaattgtgagcggataac

SEQ ID NO: 8 - DNA, 48 bp, Artificial Sequence
  Primer
  promoter 10..27: /note="promoter d"
ataagatctaaatacgccaagactagcggggaattgtgagcggataac

SEQ ID NO: 9 - DNA, 47 bp, Artificial Sequence
  Primer
  promoter 10..27: /note="promoter e"
ataagatcttcagaagtcacactataagggaattgtgagcggataac

SEQ ID NO: 10 - DNA, 47 bp, Artificial Sequence
  Primer
  promoter 10..27: /note="promoter f"
ataagatctaatagaaacatactataagggaattgtgagcggataac

SEQ ID NO: 11 - DNA, 46 bp, Artificial Sequence
  Primer
  promoter 10..26: /note="promoter h"
ataagatctaaataagactcgctaaggggaattgtgagcggataac

SEQ ID NO: 12 - DNA, 47 bp, Artificial Sequence
  Primer
  promoter 10..27: /note="promoter i"
ataagatctgattaacgtagaggataggggaattgtgagcggataac

SEQ ID NO: 13 - DNA, 47 bp, Artificial Sequence
  Primer
  promoter 10..27: /note="promoter j"
ataagatctcctcagccataactaagggggaattgtgagcggataac

SEQ ID NO: 14 - DNA, 47 bp, Artificial Sequence
  Primer
  promoter 10..27: /note="promoter k"
ataagatcttacaacactatacaataggggaattgtgagcggataac

SEQ ID NO: 15 - DNA, 17 bp, Artificial Sequence
  Primer
tccggatatagttcctc